European Patent Application EP 4 803 549 A1, published September 9, 2026. Title: 结合BCMA的抗体以及包含其的多特异性抗体. Applicant: 南京维立志博生物科技股份有限公司. The sequence listing filed with the application follows.

SEQUENCE LISTING (111 sequences)

SEQ ID NO: 1 - protein, 5 aa, synthetic construct
PSAMS

SEQ ID NO: 2 - protein, 16 aa, synthetic construct
GIYGDGRTTYADSVKG

SEQ ID NO: 3 - protein, 13 aa, synthetic construct
GIRLLSESWAQAL

SEQ ID NO: 4 - protein, 121 aa, synthetic construct
EVQVVESGGGLVQAGESLTLSCAASGFTFAPSAMSWARQPPGKEVEWVSGIYGDGRTTYADSVKGRFTISRDNAKKTVTLQMNNLEPEDSGNYICVVGIRLLSESWAQALRGQGTQVTVSS

SEQ ID NO: 5 - protein, 5 aa, synthetic construct
PSAMN

SEQ ID NO: 6 - protein, 16 aa, synthetic construct
GIYGDGKAEYADSVKG

SEQ ID NO: 7 - protein, 13 aa, synthetic construct
GIRPTDAPWAASL

SEQ ID NO: 8 - protein, 121 aa, synthetic construct
QVQLVETGGGLVQPGGSLRLSCAASGFTFSPSAMNWARQAPGKGLEWVAGIYGDGKAEYADSVKGRFTISRDNAKNMVYLQMVNLRPEDTAVYSCAVGIRPTDAPWAASLRGQGTQVTVSS

SEQ ID NO: 9 - protein, 16 aa, synthetic construct
VIYGDGRTYYADSVKG

SEQ ID NO: 10 - protein, 121 aa, synthetic construct
EVQLVESGGGLIQPGGSLRLSCAASGFTFAPSAMSWVRQPPGKGLEWVSVIYGDGRTYYADSVKGRFTISRDNSKNTLYLQMNSLRAEDTAVYYCVVGIRLLSESWAQALWGQGTLVTVSS

SEQ ID NO: 11 - protein, 228 aa, synthetic construct
EVQLVESGGGLVQPGGSLKLSCAASGFTFSTYAMNWVRQAPGKGLEWVGRIRSKYNNYATYYADSVKDRFTISRDDSKNTLYLQMNSLKTEDTAVYYCTRHGNFGNSYVSWFAYWGQGTTVTVSSASTKGPSVFPLAPSSKSTSGGTAALGCLVKDYFPEPVTVSWNSGALTSGVHTFPAVLQSSGLYSLSSVVTVPSSSLGTQTYICNVNHKPSNTKVDKKVEPKSC

SEQ ID NO: 12 - protein, 121 aa, synthetic construct
EVQVVESGGGLIQPGGSLRLSCAASGFTFAPSAMSWARQPPGKEVEWVSGIYGDGRTTYADSVKGRFTISRDNSKNTVYLQMNSLRAEDTAVYYCVVGIRLLSESWAQALRGQGTQVTVSS

SEQ ID NO: 13 - protein, 16 aa, synthetic construct
GIYGDGRTYYADSVKG

SEQ ID NO: 14 - protein, 121 aa, synthetic construct
EVQLVESGGGLIQPGGSLRLSCAASGFTFAPSAMSWARQPPGKEVEWVSGIYGDGRTYYADSVKGRFTISRDNSKNTVYLQMNSLRAEDTAVYYCVVGIRLLSESWAQALRGQGTQVTVSS

SEQ ID NO: 15 - protein, 121 aa, synthetic construct
EVQVVESGGGLIQPGGSLRLSCAASGFTFAPSAMSWARQPPGKEVEWVSGIYGDGRTTYADSVKGRFTISRDNSKNTVYLQMNSLRAEDTAVYICVVGIRLLSESWAQALRGQGTQVTVSS

SEQ ID NO: 16 - protein, 121 aa, synthetic construct
EVQLVESGGGLIQPGGSLRLSCAASGFTFAPSAMSWARQPPGKGLEWVSGIYGDGRTYYADSVKGRFTISRDNSKNTVYLQMNSLRAEDTAVYYCVVGIRLLSESWAQALRGQGTQVTVSS

SEQ ID NO: 17 - protein, 16 aa, synthetic construct
VIYGDGKAYYADSVKG

SEQ ID NO: 18 - protein, 121 aa, synthetic construct
EVQLVETGGGLIQPGGSLRLSCAASGFTFSPSAMSWVRQAPGKGLEWVSVIYGDGKAYYADSVKGRFTISRDNSKNTLYLQMNSLRAEDTAVYYCAVGIRPTDAPWAASLWGQGTLVTVSS

SEQ ID NO: 19-20 - skipped (2 entries)

SEQ ID NO: 21 - protein, 121 aa, synthetic construct
EVQLVETGGGLIQPGGSLRLSCAASGFTFSPSAMSWARQAPGKGLEWVSVIYGDGKAYYADSVKGRFTISRDNSKNTLYLQMNSLRAEDTAVYYCAVGIRPTDAPWAASLRGQGTLVTVSS

SEQ ID NO: 22 - protein, 121 aa, synthetic construct
EVQLVETGGGLIQPGGSLRLSCAASGFTFSPSAMSWARQAPGKGLEWVSGIYGDGKAEYADSVKGRFTISRDNSKNTVYLQMNSLRAEDTAVYYCAVGIRPTDAPWAASLRGQGTLVTVSS

SEQ ID NO: 23 - protein, 121 aa, synthetic construct
EVQLVETGGGLIQPGGSLRLSCAASGFTFSPSAMSWARQAPGKGLEWVSGIYGDGKAEYADSVKGRFTISRDNSKNTVYLQMNSLRAEDTAVYSCAVGIRPTDAPWAASLRGQGTLVTVSS

SEQ ID NO: 24 - protein, 5 aa, synthetic construct
ASVMS

SEQ ID NO: 25 - protein, 15 aa, synthetic construct
SMLNSNTNYADSVKG

SEQ ID NO: 26 - protein, 6 aa, synthetic construct
ERSGVY

SEQ ID NO: 27 - protein, 113 aa, synthetic construct
EVQLLESGGGLVQPGGSLRLSCAASGIFLSASVMSWYRQAPGKQRELVASMLNSNTNYADSVKGRFTISRDNSKNTMYLQMNSLRAEDTAVYYCNAERSGVYWGQGTQVTVSS

SEQ ID NO: 28 - protein, 5 aa, synthetic construct
TYAMN

SEQ ID NO: 29 - protein, 19 aa, synthetic construct
RIRSKYNNYATYYADSVKD

SEQ ID NO: 30 - protein, 14 aa, synthetic construct
HGNFGNSYVSWFAY

SEQ ID NO: 31 - protein, 14 aa, synthetic construct
RSSTGAVTTSNYAN

SEQ ID NO: 32 - protein, 7 aa, synthetic construct
GTNKRAP

SEQ ID NO: 33 - protein, 9 aa, synthetic construct
ALWYSNLWV

SEQ ID NO: 34 - protein, 125 aa, synthetic construct
EVQLVESGGGLVQPGGSLKLSCAASGFTFSTYAMNWVRQAPGKGLEWVGRIRSKYNNYATYYADSVKDRFTISRDDSKNTLYLQMNSLKTEDTAVYYCTRHGNFGNSYVSWFAYWGQGTTVTVSS

SEQ ID NO: 35 - protein, 110 aa, synthetic construct
QAVVTQEPSLTVSPGGTVTLTCRSSTGAVTTSNYANWVQQKPGQAPRGLIGGTNKRAPGVPARFSGSLLGGKAALTLSGAQPEDEAEYFCALWYSNLWVFGGGTKLTVLG

SEQ ID NO: 36 - protein, 5 aa, synthetic construct
THYMY

SEQ ID NO: 37 - protein, 17 aa, synthetic construct
GINPSNEATNFNEKFKT

SEQ ID NO: 38 - protein, 10 aa, synthetic construct
VGGLSYTMDY

SEQ ID NO: 39 - protein, 17 aa, synthetic construct
KSSQSLLYSSNQKNYLA

SEQ ID NO: 40 - protein, 7 aa, synthetic construct
WASTRES

SEQ ID NO: 41 - protein, 9 aa, synthetic construct
QQYYSYPRT

SEQ ID NO: 42 - protein, 119 aa, synthetic construct
QVQLVQSGAEVKKPGASVKVSCKASGYTFTTHYMYWVRQAPGQGLEWIGGINPSNEATNFNEKFKTKATLTVDKSTSTAYMELSSLRSEDTAVYYCTRVGGLSYTMDYWGQGTLVTVSS

SEQ ID NO: 43 - protein, 113 aa, synthetic construct
DIVMTQSPDSLAVSLGERVTMNCKSSQSLLYSSNQKNYLAWYQQKPGQPPKLLIYWASTRESGVPDRFSGSGYGTDFTLTISSLQAEDVAVYYCQQYYSYPRTFGGGTKLEIK

SEQ ID NO: 44 - protein, 353 aa, synthetic construct
EVQVVESGGGLVQAGESLTLSCAASGFTFAPSAMSWARQPPGKEVEWVSGIYGDGRTTYADSVKGRFTISRDNAKKTVTLQMNNLEPEDSGNYICVVGIRLLSESWAQALRGQGTQVTVSSEPKSSDKTHTCPPCPAPEAAGGPSVFLFPPKPKDTLMISRTPEVTCVVVAVSHEDPEVKFNWYVDGVEVHNAKTKPREEQYNSTYRVVSVLTVLHQDWLNGKEYKCKVSNKALAAPIEKTISKAKGQPREPQVYTLPPSRDELTKNQVSLTCLVKGFYPSDIAVEWESNGQPENNYKTTPPVLDSDGSFFLYSKLTVDKSRWQQGNVFSCSVMHEALHNHYTQKSLSLSPGK

SEQ ID NO: 45 - protein, 353 aa, synthetic construct
QVQLVETGGGLVQPGGSLRLSCAASGFTFSPSAMNWARQAPGKGLEWVAGIYGDGKAEYADSVKGRFTISRDNAKNMVYLQMVNLRPEDTAVYSCAVGIRPTDAPWAASLRGQGTQVTVSSEPKSSDKTHTCPPCPAPEAAGGPSVFLFPPKPKDTLMISRTPEVTCVVVAVSHEDPEVKFNWYVDGVEVHNAKTKPREEQYNSTYRVVSVLTVLHQDWLNGKEYKCKVSNKALAAPIEKTISKAKGQPREPQVYTLPPSRDELTKNQVSLTCLVKGFYPSDIAVEWESNGQPENNYKTTPPVLDSDGSFFLYSKLTVDKSRWQQGNVFSCSVMHEALHNHYTQKSLSLSPGK

SEQ ID NO: 46 - protein, 353 aa, synthetic construct
EVQLVESGGGLIQPGGSLRLSCAASGFTFAPSAMSWVRQPPGKGLEWVSVIYGDGRTYYADSVKGRFTISRDNSKNTLYLQMNSLRAEDTAVYYCVVGIRLLSESWAQALWGQGTLVTVSSEPKSSDKTHTCPPCPAPEAAGGPSVFLFPPKPKDTLMISRTPEVTCVVVAVSHEDPEVKFNWYVDGVEVHNAKTKPREEQYNSTYRVVSVLTVLHQDWLNGKEYKCKVSNKALAAPIEKTISKAKGQPREPQVYTLPPSRDELTKNQVSLTCLVKGFYPSDIAVEWESNGQPENNYKTTPPVLDSDGSFFLYSKLTVDKSRWQQGNVFSCSVMHEALHNHYTQKSLSLSPGK

SEQ ID NO: 47 - protein, 232 aa, synthetic construct
EPKSSDKTHTCPPCPAPEAAGGPSVFLFPPKPKDTLMISRTPEVTCVVVAVSHEDPEVKFNWYVDGVEVHNAKTKPREEQYNSTYRVVSVLTVLHQDWLNGKEYKCKVSNKALAAPIEKTISKAKGQPREPQVYTLPPCRDELTKNQVSLWCLVKGFYPSDIAVEWESNGQPENNYKTTPPVLDSDGSFFLYSKLTVDKSRWQQGNVFSCSVMHEALHNHYTQKSLSLSPGK

SEQ ID NO: 48 - protein, 353 aa, synthetic construct
EVQVVESGGGLIQPGGSLRLSCAASGFTFAPSAMSWARQPPGKEVEWVSGIYGDGRTTYADSVKGRFTISRDNSKNTVYLQMNSLRAEDTAVYYCVVGIRLLSESWAQALRGQGTQVTVSSEPKSSDKTHTCPPCPAPEAAGGPSVFLFPPKPKDTLMISRTPEVTCVVVAVSHEDPEVKFNWYVDGVEVHNAKTKPREEQYNSTYRVVSVLTVLHQDWLNGKEYKCKVSNKALAAPIEKTISKAKGQPREPQVYTLPPSRDELTKNQVSLTCLVKGFYPSDIAVEWESNGQPENNYKTTPPVLDSDGSFFLYSKLTVDKSRWQQGNVFSCSVMHEALHNHYTQKSLSLSPGK

SEQ ID NO: 49 - protein, 353 aa, synthetic construct
EVQLVESGGGLIQPGGSLRLSCAASGFTFAPSAMSWARQPPGKEVEWVSGIYGDGRTYYADSVKGRFTISRDNSKNTVYLQMNSLRAEDTAVYYCVVGIRLLSESWAQALRGQGTQVTVSSEPKSSDKTHTCPPCPAPEAAGGPSVFLFPPKPKDTLMISRTPEVTCVVVAVSHEDPEVKFNWYVDGVEVHNAKTKPREEQYNSTYRVVSVLTVLHQDWLNGKEYKCKVSNKALAAPIEKTISKAKGQPREPQVYTLPPSRDELTKNQVSLTCLVKGFYPSDIAVEWESNGQPENNYKTTPPVLDSDGSFFLYSKLTVDKSRWQQGNVFSCSVMHEALHNHYTQKSLSLSPGK

SEQ ID NO: 50 - protein, 353 aa, synthetic construct
EVQVVESGGGLIQPGGSLRLSCAASGFTFAPSAMSWARQPPGKEVEWVSGIYGDGRTTYADSVKGRFTISRDNSKNTVYLQMNSLRAEDTAVYICVVGIRLLSESWAQALRGQGTQVTVSSEPKSSDKTHTCPPCPAPEAAGGPSVFLFPPKPKDTLMISRTPEVTCVVVAVSHEDPEVKFNWYVDGVEVHNAKTKPREEQYNSTYRVVSVLTVLHQDWLNGKEYKCKVSNKALAAPIEKTISKAKGQPREPQVYTLPPSRDELTKNQVSLTCLVKGFYPSDIAVEWESNGQPENNYKTTPPVLDSDGSFFLYSKLTVDKSRWQQGNVFSCSVMHEALHNHYTQKSLSLSPGK

SEQ ID NO: 51 - protein, 353 aa, synthetic construct
EVQLVESGGGLIQPGGSLRLSCAASGFTFAPSAMSWARQPPGKGLEWVSGIYGDGRTYYADSVKGRFTISRDNSKNTVYLQMNSLRAEDTAVYYCVVGIRLLSESWAQALRGQGTQVTVSSEPKSSDKTHTCPPCPAPEAAGGPSVFLFPPKPKDTLMISRTPEVTCVVVAVSHEDPEVKFNWYVDGVEVHNAKTKPREEQYNSTYRVVSVLTVLHQDWLNGKEYKCKVSNKALAAPIEKTISKAKGQPREPQVYTLPPSRDELTKNQVSLTCLVKGFYPSDIAVEWESNGQPENNYKTTPPVLDSDGSFFLYSKLTVDKSRWQQGNVFSCSVMHEALHNHYTQKSLSLSPGK

SEQ ID NO: 52 - protein, 353 aa, synthetic construct
EVQLVETGGGLIQPGGSLRLSCAASGFTFSPSAMSWVRQAPGKGLEWVSVIYGDGKAYYADSVKGRFTISRDNSKNTLYLQMNSLRAEDTAVYYCAVGIRPTDAPWAASLWGQGTLVTVSSEPKSSDKTHTCPPCPAPEAAGGPSVFLFPPKPKDTLMISRTPEVTCVVVAVSHEDPEVKFNWYVDGVEVHNAKTKPREEQYNSTYRVVSVLTVLHQDWLNGKEYKCKVSNKALAAPIEKTISKAKGQPREPQVYTLPPSRDELTKNQVSLTCLVKGFYPSDIAVEWESNGQPENNYKTTPPVLDSDGSFFLYSKLTVDKSRWQQGNVFSCSVMHEALHNHYTQKSLSLSPGK

SEQ ID NO: 53 - protein, 353 aa, synthetic construct
EVQLVETGGGLIQPGGSLRLSCAASGFTFSPSAMSWARQAPGKGLEWVSVIYGDGKAYYADSVKGRFTISRDNSKNTLYLQMNSLRAEDTAVYYCAVGIRPTDAPWAASLRGQGTLVTVSSEPKSSDKTHTCPPCPAPEAAGGPSVFLFPPKPKDTLMISRTPEVTCVVVAVSHEDPEVKFNWYVDGVEVHNAKTKPREEQYNSTYRVVSVLTVLHQDWLNGKEYKCKVSNKALAAPIEKTISKAKGQPREPQVYTLPPSRDELTKNQVSLTCLVKGFYPSDIAVEWESNGQPENNYKTTPPVLDSDGSFFLYSKLTVDKSRWQQGNVFSCSVMHEALHNHYTQKSLSLSPGK

SEQ ID NO: 54 - protein, 353 aa, synthetic construct
EVQLVETGGGLIQPGGSLRLSCAASGFTFSPSAMSWARQAPGKGLEWVSGIYGDGKAEYADSVKGRFTISRDNSKNTVYLQMNSLRAEDTAVYYCAVGIRPTDAPWAASLRGQGTLVTVSSEPKSSDKTHTCPPCPAPEAAGGPSVFLFPPKPKDTLMISRTPEVTCVVVAVSHEDPEVKFNWYVDGVEVHNAKTKPREEQYNSTYRVVSVLTVLHQDWLNGKEYKCKVSNKALAAPIEKTISKAKGQPREPQVYTLPPSRDELTKNQVSLTCLVKGFYPSDIAVEWESNGQPENNYKTTPPVLDSDGSFFLYSKLTVDKSRWQQGNVFSCSVMHEALHNHYTQKSLSLSPGK

SEQ ID NO: 55 - protein, 353 aa, synthetic construct
EVQLVETGGGLIQPGGSLRLSCAASGFTFSPSAMSWARQAPGKGLEWVSGIYGDGKAEYADSVKGRFTISRDNSKNTVYLQMNSLRAEDTAVYSCAVGIRPTDAPWAASLRGQGTLVTVSSEPKSSDKTHTCPPCPAPEAAGGPSVFLFPPKPKDTLMISRTPEVTCVVVAVSHEDPEVKFNWYVDGVEVHNAKTKPREEQYNSTYRVVSVLTVLHQDWLNGKEYKCKVSNKALAAPIEKTISKAKGQPREPQVYTLPPSRDELTKNQVSLTCLVKGFYPSDIAVEWESNGQPENNYKTTPPVLDSDGSFFLYSKLTVDKSRWQQGNVFSCSVMHEALHNHYTQKSLSLSPGK

SEQ ID NO: 56 - protein, 353 aa, synthetic construct
EVQVVESGGGLIQPGGSLRLSCAASGFTFAPSAMSWARQPPGKEVEWVSGIYGDGRTTYADSVKGRFTISRDNSKNTVYLQMNSLRAEDTAVYYCVVGIRLLSESWAQALRGQGTQVTVSSEPKSSDKTHTCPPCPAPEAAGGPSVFLFPPKPKDTLMISRTPEVTCVVVAVSHEDPEVKFNWYVDGVEVHNAKTKPREEQYNSTYRVVSVLTVLHQDWLNGKEYKCKVSNKALAAPIEKTISKAKGQPREPQVCTLPPSRDELTKNQVSLSCAVKGFYPSDIAVEWESNGQPENNYKTTPPVLDSDGSFFLVSKLTVDKSRWQQGNVFSCSVMHEALHNHYTQKSLSLSPGK

SEQ ID NO: 57 - protein, 482 aa, synthetic construct
EVQLVESGGGLVQPGGSLKLSCAASGFTFSTYAMNWVRQAPGKGLEWVGRIRSKYNNYATYYADSVKDRFTISRDDSKNTLYLQMNSLKTEDTAVYYCTRHGNFGNSYVSWFAYWGQGTTVTVSSGGGGSGGGGSGGGGSQAVVTQEPSLTVSPGGTVTLTCRSSTGAVTTSNYANWVQQKPGQAPRGLIGGTNKRAPGVPARFSGSLLGGKAALTLSGAQPEDEAEYFCALWYSNLWVFGGGTKLTVLGEPKSSDKTHTCPPCPAPEAAGGPSVFLFPPKPKDTLMISRTPEVTCVVVAVSHEDPEVKFNWYVDGVEVHNAKTKPREEQYNSTYRVVSVLTVLHQDWLNGKEYKCKVSNKALAAPIEKTISKAKGQPREPQVYTLPPCRDELTKNQVSLWCLVKGFYPSDIAVEWESNGQPENNYKTTPPVLDSDGSFFLYSKLTVDKSRWQQGNVFSCSVMHEALHNHYTQKSLSLSPGK

SEQ ID NO: 58 - protein, 471 aa, synthetic construct
EVQLLESGGGLVQPGGSLRLSCAASGIFLSASVMSWYRQAPGKQRELVASMLNSNTNYADSVKGRFTISRDNSKNTMYLQMNSLRAEDTAVYYCNAERSGVYWGQGTQVTVSSGGSGGEVQVVESGGGLIQPGGSLRLSCAASGFTFAPSAMSWARQPPGKEVEWVSGIYGDGRTTYADSVKGRFTISRDNSKNTVYLQMNSLRAEDTAVYYCVVGIRLLSESWAQALRGQGTQVTVSSEPKSSDKTHTCPPCPAPEAAGGPSVFLFPPKPKDTLMISRTPEVTCVVVAVSHEDPEVKFNWYVDGVEVHNAKTKPREEQYNSTYRVVSVLTVLHQDWLNGKEYKCKVSNKALAAPIEKTISKAKGQPREPQVCTLPPSRDELTKNQVSLSCAVKGFYPSDIAVEWESNGQPENNYKTTPPVLDSDGSFFLVSKLTVDKSRWQQGNVFSCSVMHEALHNHYTQKSLSLSPGK

SEQ ID NO: 59 - protein, 455 aa, synthetic construct
EVQLVESGGGLVQPGGSLKLSCAASGFTFSTYAMNWVRQAPGKGLEWVGRIRSKYNNYATYYADSVKDRFTISRDDSKNTLYLQMNSLKTEDTAVYYCTRHGNFGNSYVSWFAYWGQGTTVTVSSASTKGPSVFPLAPSSKSTSGGTAALGCLVKDYFPEPVTVSWNSGALTSGVHTFPAVLQSSGLYSLSSVVTVPSSSLGTQTYICNVNHKPSNTKVDKKVEPKSCDKTHTCPPCPAPEAAGGPSVFLFPPKPKDTLMISRTPEVTCVVVAVSHEDPEVKFNWYVDGVEVHNAKTKPREEQYNSTYRVVSVLTVLHQDWLNGKEYKCKVSNKALAAPIEKTISKAKGQPREPQVYTLPPCRDELTKNQVSLWCLVKGFYPSDIAVEWESNGQPENNYKTTPPVLDSDGSFFLYSKLTVDKSRWQQGNVFSCSVMHEALHNHYTQKSLSLSPGK

SEQ ID NO: 60 - protein, 214 aa, synthetic construct
QAVVTQEPSLTVSPGGTVTLTCRSSTGAVTTSNYANWVQQKPGQAPRGLIGGTNKRAPGVPARFSGSLLGGKAALTLSGAQPEDEAEYFCALWYSNLWVFGGGTKLTVLGQPKAAPSVTLFPPSSEELQANKATLVCLISDFYPGAVTVAWKADSSPVKAGVETTTPSKQSNNKYAASSYLSLTPEQWKSHRSYSCQVTHEGSTVEKTVAPTEC

SEQ ID NO: 61 - protein, 709 aa, synthetic construct
QVQLVQSGAEVKKPGASVKVSCKASGYTFTTHYMYWVRQAPGQGLEWIGGINPSNEATNFNEKFKTKATLTVDKSTSTAYMELSSLRSEDTAVYYCTRVGGLSYTMDYWGQGTLVTVSSASTKGPSVFPLAPSSKSTSGGTAALGCLVKDYFPEPVTVSWNSGALTSGVHTFPAVLQSSGLYSLSSVVTVPSSSLGTQTYICNVNHKPSNTKVDKKVEPKSCGGGGSEVQLVESGGGLVQPGGSLKLSCAASGFTFSTYAMNWVRQAPGKGLEWVGRIRSKYNNYATYYADSVKDRFTISRDDSKNTLYLQMNSLKTEDTAVYYCTRHGNFGNSYVSWFAYWGQGTTVTVSSGGGGSGGGGSGGGGSQAVVTQEPSLTVSPGGTVTLTCRSSTGAVTTSNYANWVQQKPGQAPRGLIGGTNKRAPGVPARFSGSLLGGKAALTLSGAQPEDEAEYFCALWYSNLWVFGGGTKLTVLGEPKSSDKTHTCPPCPAPEAAGGPSVFLFPPKPKDTLMISRTPEVTCVVVAVSHEDPEVKFNWYVDGVEVHNAKTKPREEQYNSTYRVVSVLTVLHQDWLNGKEYKCKVSNKALAAPIEKTISKAKGQPREPQVYTLPPCRDELTKNQVSLWCLVKGFYPSDIAVEWESNGQPENNYKTTPPVLDSDGSFFLYSKLTVDKSRWQQGNVFSCSVMHEALHNHYTQKSLSLSPGK

SEQ ID NO: 62 - protein, 220 aa, synthetic construct
DIVMTQSPDSLAVSLGERVTMNCKSSQSLLYSSNQKNYLAWYQQKPGQPPKLLIYWASTRESGVPDRFSGSGYGTDFTLTISSLQAEDVAVYYCQQYYSYPRTFGGGTKLEIKRTVAAPSVFIFPPSDEQLKSGTASVVCLLNNFYPREAKVQWKVDNALQSGNSQESVTEQDSKDSTYSLSSTLTLSKADYEKHKVYACEVTHQGLSSPVTKSFNRGEC

SEQ ID NO: 63 - protein, 448 aa, synthetic construct
QLQLQESGPGLVKPSETLSLTCTVSGGSISSGSYFWGWIRQPPGKGLEWIGSIYYSGITYYNPSLKSRVTISVDTSKNQFSLKLSSVTAADTAVYYCARHDGAVAGLFDYWGQGTLVTVSSASTKGPSVFPLAPCSRSTSESTAALGCLVKDYFPEPVTVSWNSGALTSGVHTFPAVLQSSGLYSLSSVVTVPSSSLGTKTYTCNVDHKPSNTKVDKRVESKYGPPCPPCPAPEAAGGPSVFLFPPKPKDTLMISRTPEVTCVVVDVSQEDPEVQFNWYVDGVEVHNAKTKPREEQFNSTYRVVSVLTVLHQDWLNGKEYKCKVSNKGLPSSIEKTISKAKGQPREPQVYTLPPSQEEMTKNQVSLTCLVKGFYPSDIAVEWESNGQPENNYKTTPPVLDSDGSFFLYSRLTVDKSRWQEGNVFSCSVMHEALHNHYTQKSLSLSLGK

SEQ ID NO: 64 - protein, 213 aa, synthetic construct
SYVLTQPPSVSVAPGQTARITCGGNNIGSKSVHWYQQPPGQAPVVVVYDDSDRPSGIPERFSGSNSGNTATLTISRVEAGDEAVYYCQVWDSSSDHVVFGGGTKLTVLGQPKAAPSVTLFPPSSEELQANKATLVCLISDFYPGAVTVAWKGDSSPVKAGVETTTPSKQSNNKYAASSYLSLTPEQWKSHRSYSCQVTHEGSTVEKTVAPTEC

SEQ ID NO: 65 - protein, 452 aa, synthetic construct
EVQLVESGGGLVQPGGSLRLSCAASGFTFNTYAMNWVRQAPGKGLEWVARIRSKYNNYATYYAASVKGRFTISRDDSKNSLYLQMNSLKTEDTAVYYCARHGNFGNSYVSWFAYWGQGTLVTVSSASTKGPSVFPLAPCSRSTSESTAALGCLVKDYFPEPVTVSWNSGALTSGVHTFPAVLQSSGLYSLSSVVTVPSSSLGTKTYTCNVDHKPSNTKVDKRVESKYGPPCPPCPAPEAAGGPSVFLFPPKPKDTLMISRTPEVTCVVVDVSQEDPEVQFNWYVDGVEVHNAKTKPREEQFNSTYRVVSVLTVLHQDWLNGKEYKCKVSNKGLPSSIEKTISKAKGQPREPQVYTLPPSQEEMTKNQVSLTCLVKGFYPSDIAVEWESNGQPENNYKTTPPVLDSDGSFLLYSKLTVDKSRWQEGNVFSCSVMHEALHNHYTQKSLSLSLGK

SEQ ID NO: 66 - protein, 214 aa, synthetic construct
QTVVTQEPSLTVSPGGTVTLTCRSSTGAVTTSNYANWVQQKPGQAPRGLIGGTNKRAPGTPARFSGSLLGGKAALTLSGVQPEDEAEYYCALWYSNLWVFGGGTKLTVLGQPKAAPSVTLFPPSSEELQANKATLVCLISDFYPGAVTVAWKADSSPVKAGVETTTPSKQSNNKYAASSYLSLTPEQWKSHRSYSCQVTHEGSTVEKTVAPTEC

SEQ ID NO: 67 - protein, 445 aa, synthetic construct
QVQLVQSGAEVKKPGASVKVSCKASGYSFTGYTMNWVRQAPGQGLEWMGLINPYNSDTNYAQKLQGRVTMTTDTSTSTAYMELRSLRSDDTAVYYCARVALRVALDYWGQGTLVTVSSASTKGPSVFPLAPCSRSTSESTAALGCLVKDYFPEPVTVSWNSGALTSGVHTFPAVLQSSGLYSLSSVVTVPSSSLGTKTYTCNVDHKPSNTKVDKRVESKYGPPCPPCPAPEAAGGPSVFLFPPKPKDTLMISRTPEVTCVVVDVSQEDPEVQFNWYVDGVEVHNAKTKPREEQFNSTYRVVSVLTVLHQDWLNGKEYKCKVSNKGLPSSIEKTISKAKGQPREPQVYTLPPSQEEMTKNQVSLTCLVKGFYPSDIAVEWESNGQPENNYKTTPPVLDSDGSFFLYSRLTVDKSRWQEGNVFSCSVMHEALHNHYTQKSLSLSLGK

SEQ ID NO: 68 - protein, 214 aa, synthetic construct
DIQMTQSPSSLSASVGDRVTITCKASQNVATHVGWYQQKPGKAPKRLIYSASYRYSGVPSRFSGSGSGTEFTLTISNLQPEDFATYYCQQYNRYPYTFGQGTKLEIKRTVAAPSVFIFPPSDEQLKSGTASVVCLLNNFYPREAKVQWKVDNALQSGNSQESVTEQDSKDSTYSLSSTLTLSKADYEKHKVYACEVTHQGLSSPVTKSFNRGEC

SEQ ID NO: 69 - protein, 721 aa, synthetic construct
QVQLQQSGPRLVRPSQTLSLTCAISGDSVFNNNAAWSWIRQSPSRGLEWLGRTYYRSKWLYDYAVSVKSRITVNPDTSRNQFTLQLNSVTPEDTALYYCARGYSSSFDYWGQGTLVTVSSASTKGPSVFPLAPSSKSTSGGTAALGCLVKDYFPEPVTVSWNSGALTSGVHTFPAVLQSSGLYSLSSVVTVPSSSLGTQTYICNVNHKPSNTKVDKKVEPKSCDKTHTCPPCPAPEAAGGPSVFLFPPKPKDTLMISRTPEVTCVVVSVSHEDPEVKFNWYVDGVEVHNAKTKPREEQYNSTYRVVSVLTVLHQDWLNGKEYKCKVSNKALPAPIEKTISKAKGQPREPQVYTLPPSREEMTKNQVSLSCAVKGFYPSDIAVEWESNGQPENNYKTTPPVLDSDGSFFLVSKLTVDKSRWQQGNVFSCSVMHEALHNRFTQKSLSLSPGKGGGGSGGGGSGGGGSGGGGSDIVMTQTPLSSPVTLGQPASISCRSSQSLVHSDGNTYLSWLQQRPGQPPRLLIYKISNRFFGVPDRFSGSGAGTDFTLKISRVEAEDVGVYYCMQATQFPHTFGQGTKLEIKGGSEGKSSGSGSESKSTGGSQVTLKESGPVLVKPTETLTLTCTVSGFSLTNIRMSVSWIRQPPGKALEWLAHIFSNDEKSYSTSLKSRLTISRDTSKSQVVLTLTNVDPVDTATYYCARMRLPYGMDVWGQGTTVTVSS

SEQ ID NO: 70 - protein, 484 aa, synthetic construct
EIVLTQSPGTLSLSPGERATLSCRASQSISSSFLTWYQQKPGQAPRLLIYGASSRATGIPDRFSGGGSGTDFTLTISRLEPEDFAVYYCQHYGSSPMYTFGQGTKLEIKGGSEGKSSGSGSESKSTGGSEVQLLESGGGLVQPGGSLRLSCAASGFTFSSYAMSWVRQAPGKGLEWVSAISGSGGSTYYADSVKGRFTISRDNSKNTLYLQMNSLRAEDTAVYYCAKDEGYSSGHYYGMDVWGQGTTVTVSSEPKSSDKTHTCPPCPAPEAAGGPSVFLFPPKPKDTLMISRTPEVTCVVVSVSHEDPEVKFNWYVDGVEVHNAKTKPREEQYNSTYRVVSVLTVLHQDWLNGKEYKCKVSNKALPAPIEKTISKAKGQPREPQVYTLPPSREEMTKNQVSLWCLVKGFYPSDIAVEWESNGQPENNYKTTPPVLDSDGSFFLYSKLTVDKSRWQQGNVFSCSVMHEALHNHYTQKSLSLSPGK

SEQ ID NO: 71 - protein, 214 aa, synthetic construct
ALTQPASVSGSPGQSITISCTGTSSNIGTYKFVSWYQQHPDKAPKVLLYEVSKRPSGVSSRFSGSKSGNTASLTISGLQAEDQADYHCVSYAGSGTLLFGGGTKLTVLGQPKAAPSVTLFPPSSEELQANKATLVCLISDFYPGAVTVAWKADSSPVKAGVETTTPSKQSNNKYAASSYLSLTPEQWKSHRSYSCQVTHEGSTVEKTVAPTECS

SEQ ID NO: 72 - protein, 450 aa, synthetic construct
QVQLVQSGAEVKKPGASVKVSCKASGYTFIGYVMHWVRQAPGQGLEWMGYINPYNDVSQHQGKFKGRVTMTSDTSTSTVYMELSSLRSEDTAVYYCAREGRLGLRVLAYWGQGTLVTVSSASTKGPSVFPLAPSSKSTSGGTAALGCLVKDYFPEPVTVSWNSGALTSGVHTFPAVLQSSGLYSLSSVVTVPSSSLGTQTYICNVNHKPSNTKVDKKVEPKSCDKTHTCPPCPAPEAAGGPSVFLFPPKPKDTLMISRTPEVTCVVVDVSHEDPEVKFNWYVDGVEVHNAKTKPREEQYNSTYRVVSVLTVLHQDWLNGKEYKCKVSNKALPAPIEKTISKAKGQPREPQVYTLPPSRDELTKNQVSLWCLVKGFYPSDIAVEWESNGQPENNYKTTPPVLDSDGSFFLYSKLTVDKSRWQQGNVFSCSVMHEALHNHYTQKSLSLSPGK

SEQ ID NO: 73 - protein, 711 aa, synthetic construct
EVQLVESGGGLVQPGGSLKLSCAASGFTFNTYAMNWVRQASGKGLEWVGRIRSKYNNYATYYADSVKDRFTISRDDSKSTLYLQMNSLKTEDTAVYYCARHGNFGQSYVSWFAYWGQGTTVTVSSASTKGPSVFPLAPSSKSTSGGTAALGCLVKDYFPEPVTVSWNSGALTSGVHTFPAVLQSSGLYSLSSVVTVPSSSLGTQTYICNVNHKPSNTKVDKKVEPKSSDKTHTCPPCPAPEAAGGPSVFLFPPKPKDTLMISRTPEVTCVVVDVSHEDPEVKFNWYVDGVEVHNAKTKPREEQYNSTYRVVSVLTVLHQDWLNGKEYKCKVSNKALPAPIEKTISKAKGQPREPQVYTLPPSRDELTKNQVSLSCAVKGFYPSDIAVEWESNGQPENNYKTTPPVLDSDGSFFLVSKLTVDKSRWQQGNVFSCSVMHEALHNHYTQKSLSLSPGKGGGGSGGGGSEIVLTQSPATLSLSPGERATLSCRASQSVSSYLAWYQQKPGQAPRLLIYDASKRATGIPARFSGSGSGTDFTLTISSLEPEDFAVYYCQQASALPLTFGCGTKVEIKGGGGSGGGGSGGGGSEVQLVESGGGLVQPGRSLRLSCAASGFTFGDYAIHWVRQAPGKCLEWVSGISWDSSSIAYADSVKGRFTISRDNAKNSLYLQMNSLRAEDTAVYYCAKDSPVRDSFGSIAFDIWGQGTMVTVSS

SEQ ID NO: 74 - protein, 214 aa, synthetic construct
QAVVTQEPSLTVSPGGTVTLTCRSSTGAVTTSNYANWVQQKPGQAPRGLIGGTNKRAPGVPARFSGSLLGDKAALTLLGAQPEDEAEYYCALWYSNLWVFGQGTKLTVLGQPKAAPSVTLFPPSSEELQANKATLVCLISDFYPGAVTVAWKADSSPVKAGVETTTPSKQSNNKYAASSYLSLTPEQWKSHRSYSCQVTHEGSTVEKTVAPTEC

SEQ ID NO: 75 - protein, 218 aa, synthetic construct
DIVMTQSPDSLAVSLGERATINCRASESVDSYGITFMNWYQQKPGQPPKLLIYAASNQGSGVPDRFSGSGSGTDFTLTISSLQAEDVAVYYCQQSKEVPWTFGQGTKLEIKRTVAAPSVFIFPPSDEQLKSGTASVVCLLNNFYPREAKVQWKVDNALQSGNSQESVTEQDSKDSTYSLSSTLTLSKADYEKHKVYACEVTHQGLSSPVTKSFNRGEC

SEQ ID NO: 76 - protein, 351 aa, synthetic construct
DVQLVESGGGLVQPGGSLRLSCAASGRTFSSIVMGWFRQAPGKEREFVGAIMWNDGITYLQDSVKGRFTIFRDNAKNTVYLQMNSLKLEDTAVYYCAASKGRYSEYEYWGQGTQVTVSSEPKSSDKTHTCPPCPAPELLGGPSVFLFPPKPKDTLMISRTPEVTCVVVDVSHEDPEVKFNWYVDGVEVHNAKTKPREEQYNSTYRVVSVLTVLHQDWLNGKEYKCKVSNKALPAPIEKTISKAKGQPREPQVYTLPPSRDELTKNQVSLTCLVKGFYPSDIAVEWESNGQPENNYKTTPPVLDSDGSFFLYSKLTVDKSRWQQGNVFSCSVMHEALHNHYTQKSLSLSPGK

SEQ ID NO: 77 - protein, 286 aa, synthetic construct
MLQMAGQCSQNEYFDSLLHACIPCQLRCSSNTPPLTCQRYCNASVTNSVKGTNAEPKSCDKTHTCPPCPAPELLGGPSVFLFPPKPKDTLMISRTPEVTCVVVDVSHEDPEVKFNWYVDGVEVHNAKTKPREEQYNSTYRVVSVLTVLHQDWLNGKEYKCKVSNKALPAPIEKTISKAKGQPREPQVYTLPPSRDELTKNQVSLTCLVKGFYPSDIAVEWESNGQPENNYKTTPPVLDSDGSFFLYSKLTVDKSRWQQGNVFSCSVMHEALHNHYTQKSLSLSPGK

SEQ ID NO: 78 - protein, 285 aa, synthetic construct
MLQMARQCSQNEYFDSLLHDCKPCQLRCSSTPPLTCQRYCNASMTNSVKGMNAEPKSCDKTHTCPPCPAPELLGGPSVFLFPPKPKDTLMISRTPEVTCVVVDVSHEDPEVKFNWYVDGVEVHNAKTKPREEQYNSTYRVVSVLTVLHQDWLNGKEYKCKVSNKALPAPIEKTISKAKGQPREPQVYTLPPSRDELTKNQVSLTCLVKGFYPSDIAVEWESNGQPENNYKTTPPVLDSDGSFFLYSKLTVDKSRWQQGNVFSCSVMHEALHNHYTQKSLSLSPGK

SEQ ID NO: 79 - protein, 60 aa, synthetic construct
MLQMAGQCSQNEYFDSLLHACIPCQLRCSSNTPPLTCQRYCNASVTNSVKGTNAHHHHHH

SEQ ID NO: 80 - protein, 232 aa, synthetic construct
EPKSSDKTHTCPPCPAPELLGGPSVFLFPPKPKDTLMISRTPEVTCVVVDVSHEDPEVKFNWYVDGVEVHNAKTKPREEQYNSTYRVVSVLTVLHQDWLNGKEYKCKVSNKALPAPIEKTISKAKGQPREPQVYTLPPSRDELTKNQVSLTCLVKGFYPSDIAVEWESNGQPENNYKTTPPVLDSDGSFFLYSKLTVDKSRWQQGNVFSCSVMHEALHNHYTQKSLSLSPGK

SEQ ID NO: 81 - protein, 357 aa, synthetic construct
MATTVPDGCRNGLKSKYYRLCDKAEAWGIVLETVATAGVVTSVAFMLTLPILVCKVQDSNRRKMLPTQFLFLLGVLGIFGLTFAFIIGLDGSTGPTRFFLFGILFSICFSCLLAHAVSLTKLVRGRKPLSLLVILGLAVGFSLVQDVIAIEYIVLTMNRTNVNVFSELSAPRRNEDFVLLLTYVLFLMALTFLMSSFTFCGSFTGWKRHGAHIYLTMLLSIAIWVAWITLLMLPDFDRRWDDTILSSALAANGWVFLLAYVSPEFWLLTKQRNPMDYPVEDAFCKPQLVKKSYGVENRAYSQEEITQGFEETGDTLYAPYSTHFQLQNQPPQKEFSIPRAHAWPSPYKDYEVKKEGS

SEQ ID NO: 82 - protein, 403 aa, synthetic construct
MFVASERKMRAHQVLTFLLLFVITSVASENASTSRGCGLDLLPQYVSLCDLDAIWGIVVEAVAGAGALITLLLMLILLVRLPFIKEKEKKSPVGLHFLFLLGTLGLFGLTFAFIIQEDETICSVRRFLWGVLFALCFSCLLSQAWRVRRLVRHGTGPAGWQLVGLALCLMLVQVIIAVEWLVLTVLRDTRPACAYEPMDFVMALIYDMVLLVVTLGLALFTLCGKFKRWKLNGAFLLITAFLSVLIWVAWMTMYLFGNVKLQQGDAWNDPTLAITLAASGWVFVIFHAIPEIHCTLLPALQENTPNYFDTSQPRMRETAFEEDVQLPRAYMENKAFSMDEHNAALRTAGFPNGSLGKRPSGSLGKRPSAPFRSNVYQPTEMAVVLNGGTIPTAPPSHTGRHLW

SEQ ID NO: 83 - protein, 441 aa, synthetic construct
MAIHKALVMCLGLPLFLFPGAWAQGHVPPGCSQGLNPLYYNLCDRSGAWGIVLEAVAGAGIVTTFVLTIILVASLPFVQDTKKRSLLGTQVFFLLGTLGLFCLVFACVVKPDFSTCASRRFLFGVLFAICFSCLAAHVFALNFLARKNHGPRGWVIFTVALLLTLVEVIINTEWLIITLVRGSGEGGPQGNSSAGWAVASPCAIANMDFVMALIYVMLLLLGAFLGAWPALCGRYKRWRKHGVFVLLTTATSVAIWVVWIVMYTYGNKQHNSPTWDDPTLAIALAANAWAFVLFYVIPEVSQVTKSSPEQSYQGDMYPTRGVGYETILKEQKGQSMFVENKAFSMDEPVAAKRPVSPYSGYNGQLLTSVYQPTEMALMHKVPSEGAYDIILPRATANSQVMGSANSTLRAEDMYSAQSHQAATPPKDGKNSQVFRNPYVWD

SEQ ID NO: 84 - protein, 227 aa, synthetic construct
DKTHTCPPCPAPEAAGGPSVFLFPPKPKDTLMISRTPEVTCVVVAVSHEDPEVKFNWYVDGVEVHNAKTKPREEQYNSTYRVVSVLTVLHQDWLNGKEYKCKVSNKALAAPIEKTISKAKGQPREPQVCTLPPSRDELTKNQVSLSCAVKGFYPSDIAVEWESNGQPENNYKTTPPVLDSDGSFFLVSKLTVDKSRWQQGNVFSCSVMHEALHNHYTQKSLSLSPGK

SEQ ID NO: 85 - protein, 232 aa, synthetic construct
EPKSSDKTHTCPPCPAPEAAGGPSVFLFPPKPKDTLMISRTPEVTCVVVAVSHEDPEVKFNWYVDGVEVHNAKTKPREEQYNSTYRVVSVLTVLHQDWLNGKEYKCKVSNKALAAPIEKTISKAKGQPREPQVCTLPPSRDELTKNQVSLSCAVKGFYPSDIAVEWESNGQPENNYKTTPPVLDSDGSFFLVSKLTVDKSRWQQGNVFSCSVMHEALHNHYTQKSLSLSPGK

SEQ ID NO: 86 - protein, 232 aa, synthetic construct
EPKSCDKTHTCPPCPAPEAAGGPSVFLFPPKPKDTLMISRTPEVTCVVVAVSHEDPEVKFNWYVDGVEVHNAKTKPREEQYNSTYRVVSVLTVLHQDWLNGKEYKCKVSNKALAAPIEKTISKAKGQPREPQVYTLPPCRDELTKNQVSLWCLVKGFYPSDIAVEWESNGQPENNYKTTPPVLDSDGSFFLYSKLTVDKSRWQQGNVFSCSVMHEALHNHYTQKSLSLSPGK

SEQ ID NO: 87 - protein, 227 aa, synthetic construct
DKTHTCPPCPAPEAAGGPSVFLFPPKPKDTLMISRTPEVTCVVVAVSHEDPEVKFNWYVDGVEVHNAKTKPREEQYNSTYRVVSVLTVLHQDWLNGKEYKCKVSNKALAAPIEKTISKAKGQPREPQVYTLPPCRDELTKNQVSLWCLVKGFYPSDIAVEWESNGQPENNYKTTPPVLDSDGSFFLYSKLTVDKSRWQQGNVFSCSVMHEALHNHYTQKSLSLSPGK

SEQ ID NO: 88 - protein, 98 aa, synthetic construct
ASTKGPSVFPLAPSSKSTSGGTAALGCLVKDYFPEPVTVSWNSGALTSGVHTFPAVLQSSGLYSLSSVVTVPSSSLGTQTYICNVNHKPSNTKVDKKV

SEQ ID NO: 89 - protein, 330 aa, synthetic construct
ASTKGPSVFPLAPSSKSTSGGTAALGCLVKDYFPEPVTVSWNSGALTSGVHTFPAVLQSSGLYSLSSVVTVPSSSLGTQTYICNVNHKPSNTKVDKKVEPKSCDKTHTCPPCPAPEAAGGPSVFLFPPKPKDTLMISRTPEVTCVVVAVSHEDPEVKFNWYVDGVEVHNAKTKPREEQYNSTYRVVSVLTVLHQDWLNGKEYKCKVSNKALAAPIEKTISKAKGQPREPQVYTLPPSRDELTKNQVSLTCLVKGFYPSDIAVEWESNGQPENNYKTTPPVLDSDGSFFLYSKLTVDKSRWQQGNVFSCSVMHEALHNHYTQKSLSLSPGK

SEQ ID NO: 90 - protein, 227 aa, synthetic construct
DKTHTCPPCPAPEAAGGPSVFLFPPKPKDTLMISRTPEVTCVVVAVSHEDPEVKFNWYVDGVEVHNAKTKPREEQYNSTYRVVSVLTVLHQDWLNGKEYKCKVSNKALAAPIEKTISKAKGQPREPQVYTLPPSRDELTKNQVSLTCLVKGFYPSDIAVEWESNGQPENNYKTTPPVLDSDGSFFLYSKLTVDKSRWQQGNVFSCSVMHEALHNHYTQKSLSLSPGK

SEQ ID NO: 91 - protein, 105 aa, synthetic construct
GQPKAAPSVTLFPPSSEELQANKATLVCLISDFYPGAVTVAWKADSSPVKAGVETTTPSKQSNNKYAASSYLSLTPEQWKSHRSYSCQVTHEGSTVEKTVAPTEC

SEQ ID NO: 92 - protein, 330 aa, synthetic construct [sequence omitted]

SEQ ID NO: 93 - protein, 107 aa, synthetic construct [sequence omitted]

SEQ ID NO: 94 - protein, 5 aa, synthetic construct
EPKSS

SEQ ID NO: 95 - protein, 20 aa, synthetic construct
GGGGSGGGGSGGGGSGGGGS

SEQ ID NO: 96 - protein, 5 aa, synthetic construct
EPKSC

SEQ ID NO: 97 - protein, 232 aa, synthetic construct
EPKSSDKTHTCPPCPAPEAAGGPSVFLFPPKPKDTLMISRTPEVTCVVVAVSHEDPEVKFNWYVDGVEVHNAKTKPREEQYNSTYRVVSVLTVLHQDWLNGKEYKCKVSNKALAAPIEKTISKAKGQPREPQVYTLPPSRDELTKNQVSLTCLVKGFYPSDIAVEWESNGQPENNYKTTPPVLDSDGSFFLYSKLTVDKSRWQQGNVFSCSVMHEALHNHYTQKSLSLSPGK

SEQ ID NO: 98 - protein, 227 aa, synthetic construct
DKTHTCPPCPAPELLGGPSVFLFPPKPKDTLMISRTPEVTCVVVDVSHEDPEVKFNWYVDGVEVHNAKTKPREEQYNSTYRVVSVLTVLHQDWLNGKEYKCKVSNKALPAPIEKTISKAKGQPREPQVYTLPPSRDELTKNQVSLTCLVKGFYPSDIAVEWESNGQPENNYKTTPPVLDSDGSFFLYSKLTVDKSRWQQGNVFSCSVMHEALHNHYTQKSLSLSPGK

SEQ ID NO: 99 - protein, 5 aa, synthetic construct
GGGGS

SEQ ID NO: 100 - protein, 15 aa, synthetic construct
GGGGSGGGGSGGGGS

SEQ ID NO: 101 - protein, 5 aa, synthetic construct
GGSGG

SEQ ID NO: 102 - protein, 353 aa, synthetic construct
EVQLVETGGGLIQPGGSLRLSCAASGFTFSPSAMSWARQAPGKGLEWVSGIYGDGKAEYADSVKGRFTISRDNSKNTVYLQMNSLRAEDTAVYSCAVGIRPTDAPWAASLRGQGTLVTVSSEPKSSDKTHTCPPCPAPEAAGGPSVFLFPPKPKDTLMISRTPEVTCVVVAVSHEDPEVKFNWYVDGVEVHNAKTKPREEQYNSTYRVVSVLTVLHQDWLNGKEYKCKVSNKALAAPIEKTISKAKGQPREPQVCTLPPSRDELTKNQVSLSCAVKGFYPSDIAVEWESNGQPENNYKTTPPVLDSDGSFFLVSKLTVDKSRWQQGNVFSCSVMHEALHNHYTQKSLSLSPGK

SEQ ID NO: 103 - protein, 479 aa, synthetic construct
EVQLVETGGGLIQPGGSLRLSCAASGFTFSPSAMSWARQAPGKGLEWVSGIYGDGKAEYADSVKGRFTISRDNSKNTVYLQMNSLRAEDTAVYSCAVGIRPTDAPWAASLRGQGTLVTVSSGGGGSEVQLVETGGGLIQPGGSLRLSCAASGFTFSPSAMSWARQAPGKGLEWVSGIYGDGKAEYADSVKGRFTISRDNSKNTVYLQMNSLRAEDTAVYSCAVGIRPTDAPWAASLRGQGTLVTVSSEPKSSDKTHTCPPCPAPEAAGGPSVFLFPPKPKDTLMISRTPEVTCVVVAVSHEDPEVKFNWYVDGVEVHNAKTKPREEQYNSTYRVVSVLTVLHQDWLNGKEYKCKVSNKALAAPIEKTISKAKGQPREPQVCTLPPSRDELTKNQVSLSCAVKGFYPSDIAVEWESNGQPENNYKTTPPVLDSDGSFFLVSKLTVDKSRWQQGNVFSCSVMHEALHNHYTQKSLSLSPGK

SEQ ID NO: 104 - protein, 479 aa, synthetic construct
EVQVVESGGGLIQPGGSLRLSCAASGFTFAPSAMSWARQPPGKEVEWVSGIYGDGRTTYADSVKGRFTISRDNSKNTVYLQMNSLRAEDTAVYYCVVGIRLLSESWAQALRGQGTQVTVSSGGGGSEVQVVESGGGLIQPGGSLRLSCAASGFTFAPSAMSWARQPPGKEVEWVSGIYGDGRTTYADSVKGRFTISRDNSKNTVYLQMNSLRAEDTAVYYCVVGIRLLSESWAQALRGQGTQVTVSSEPKSSDKTHTCPPCPAPEAAGGPSVFLFPPKPKDTLMISRTPEVTCVVVAVSHEDPEVKFNWYVDGVEVHNAKTKPREEQYNSTYRVVSVLTVLHQDWLNGKEYKCKVSNKALAAPIEKTISKAKGQPREPQVCTLPPSRDELTKNQVSLSCAVKGFYPSDIAVEWESNGQPENNYKTTPPVLDSDGSFFLVSKLTVDKSRWQQGNVFSCSVMHEALHNHYTQKSLSLSPGK

SEQ ID NO: 105 - protein, 345 aa, synthetic construct
EVQLLESGGGLVQPGGSLRLSCAASGIFLSASVMSWYRQAPGKQRELVASMLNSNTNYADSVKGRFTISRDNSKNTMYLQMNSLRAEDTAVYYCNAERSGVYWGQGTQVTVSSEPKSSDKTHTCPPCPAPELLGGPSVFLFPPKPKDTLMISRTPEVTCVVVDVSHEDPEVKFNWYVDGVEVHNAKTKPREEQYNSTYRVVSVLTVLHQDWLNGKEYKCKVSNKALPAPIEKTISKAKGQPREPQVYTLPPSRDELTKNQVSLTCLVKGFYPSDIAVEWESNGQPENNYKTTPPVLDSDGSFFLYSKLTVDKSRWQQGNVFSCSVMHEALHNHYTQKSLSLSPGK

SEQ ID NO: 106 - protein, 113 aa, synthetic construct
EVQLQESGGGLVQAGGSLRLSCAASGIFLSASVMRWYRRAPGKQRELVASMLNSNTNYADSVKGRFTISRDNTKNTMYLQMNSLKPEDTAVYYCNAERSGVYWGQGTQVTVSS

SEQ ID NO: 107 - protein, 345 aa, synthetic construct
EVQLQESGGGLVQAGGSLRLSCAASGIFLSASVMRWYRRAPGKQRELVASMLNSNTNYADSVKGRFTISRDNTKNTMYLQMNSLKPEDTAVYYCNAERSGVYWGQGTQVTVSSEPKSSDKTHTCPPCPAPELLGGPSVFLFPPKPKDTLMISRTPEVTCVVVDVSHEDPEVKFNWYVDGVEVHNAKTKPREEQYNSTYRVVSVLTVLHQDWLNGKEYKCKVSNKALPAPIEKTISKAKGQPREPQVYTLPPSRDELTKNQVSLTCLVKGFYPSDIAVEWESNGQPENNYKTTPPVLDSDGSFFLYSKLTVDKSRWQQGNVFSCSVMHEALHNHYTQKSLSLSPGK

SEQ ID NO: 108 - protein, 345 aa, Homo sapiens
MYKDCIESTGDYFLLCDAEGPWGIILESLAILGIVVTILLLLAFLFLMRKIQDCSQWNVLPTQLLFLLSVLGLFGLAFAFIIELNQQTAPVRYFLFGVLFALCFSCLLAHASNLVKLVRGCVSFSWTTILCIAIGCSLLQIIIATEYVTLIMTRGMMFVNMTPCQLNVDFVVLLVYVLFLMALTFFVSKATFCGPCENWKQHGRLIFITVLFSIIIWVVWISMLLRGNPQFQRQPQWDDPVVCIALVTNAWVFLLLYIVPELCILYRSCRQECPLQGNACPVTAYQHSFQVENQELSRARDSDGAEEDVALTSYGTPIQPQTVDPTQECFIPQAKLSPQQDAGGV

SEQ ID NO: 109 - protein, 250 aa, synthetic construct
EVQLVESGGGLVQPGGSLKLSCAASGFTFSTYAMNWVRQAPGKGLEWVGRIRSKYNNYATYYADSVKDRFTISRDDSKNTLYLQMNSLKTEDTAVYYCTRHGNFGNSYVSWFAYWGQGTTVTVSSGGGGSGGGGSGGGGSQAVVTQEPSLTVSPGGTVTLTCRSSTGAVTTSNYANWVQQKPGQAPRGLIGGTNKRAPGVPARFSGSLLGGKAALTLSGAQPEDEAEYFCALWYSNLWVFGGGTKLTVLG

SEQ ID NO: 110 - protein, 222 aa, synthetic construct
QVQLVQSGAEVKKPGASVKVSCKASGYTFTTHYMYWVRQAPGQGLEWIGGINPSNEATNFNEKFKTKATLTVDKSTSTAYMELSSLRSEDTAVYYCTRVGGLSYTMDYWGQGTLVTVSSASTKGPSVFPLAPSSKSTSGGTAALGCLVKDYFPEPVTVSWNSGALTSGVHTFPAVLQSSGLYSLSSVVTVPSSSLGTQTYICNVNHKPSNTKVDKKVEPKSC

SEQ ID NO: 111 - protein, 232 aa, synthetic construct
EPKSCDKTHTCPPCPAPEAAGGPSVFLFPPKPKDTLMISRTPEVTCVVVAVSHEDPEVKFNWYVDGVEVHNAKTKPREEQYNSTYRVVSVLTVLHQDWLNGKEYKCKVSNKALAAPIEKTISKAKGQPREPQVCTLPPSRDELTKNQVSLSCAVKGFYPSDIAVEWESNGQPENNYKTTPPVLDSDGSFFLVSKLTVDKSRWQQGNVFSCSVMHEALHNHYTQKSLSLSPGK